European Patent Application EP 4 745 237 A1, published May 20, 2026. Title: 用于抑制己酮糖激酶表达的RNAi剂及其应用. Applicant: 云合智药（苏州）生物科技有限公司. The sequence listing filed with the application follows.

SEQUENCE LISTING (153 sequences)

SEQ ID NO: 1 - RNA, 19 nt, synthetic construct
  source 1..19: mol_type = other RNA
agttcaagtggatccacat

SEQ ID NO: 2 - RNA, 19 nt, synthetic construct
  source 1..19: mol_type = other RNA
tgcagagcctcagagcaaa

SEQ ID NO: 3 - RNA, 19 nt, synthetic construct
  source 1..19: mol_type = other RNA
cgtgcaggaagcactgaga

SEQ ID NO: 4 - RNA, 19 nt, synthetic construct
  source 1..19: mol_type = other RNA
tgctccactcggatgcttt

SEQ ID NO: 5 - RNA, 19 nt, synthetic construct
  source 1..19: mol_type = other RNA
ttgctccactcggatgctt

SEQ ID NO: 6 - RNA, 19 nt, synthetic construct
  source 1..19: mol_type = other RNA
atggcaaattgctccacta

SEQ ID NO: 7 - RNA, 19 nt, synthetic construct
  source 1..19: mol_type = other RNA
cggagcaggtgaagatgct

SEQ ID NO: 8 - RNA, 19 nt, synthetic construct
  source 1..19: mol_type = other RNA
catcggagcaggtgaagat

SEQ ID NO: 9 - RNA, 19 nt, synthetic construct
  source 1..19: mol_type = other RNA
tgacccagttcaagtggat

SEQ ID NO: 10 - RNA, 19 nt, synthetic construct
  source 1..19: mol_type = other RNA
ctgacccagttcaagtgga

SEQ ID NO: 11 - RNA, 19 nt, synthetic construct
  source 1..19: mol_type = other RNA
atctgacccagttcaagta

SEQ ID NO: 12 - RNA, 19 nt, synthetic construct
  source 1..19: mol_type = other RNA
ttgatctgacccagttcaa

SEQ ID NO: 13 - RNA, 19 nt, synthetic construct
  source 1..19: mol_type = other RNA
gttgatctgacccagttca

SEQ ID NO: 14 - RNA, 19 nt, synthetic construct
  source 1..19: mol_type = other RNA
ctgctacagactttgagaa

SEQ ID NO: 15 - RNA, 19 nt, synthetic construct
  source 1..19: mol_type = other RNA
tctgctacagactttgaga

SEQ ID NO: 16 - RNA, 19 nt, synthetic construct
  source 1..19: mol_type = other RNA
tgtctgctacagactttga

SEQ ID NO: 17 - RNA, 19 nt, synthetic construct
  source 1..19: mol_type = other RNA
gtgtctgctacagacttta

SEQ ID NO: 18 - RNA, 19 nt, synthetic construct
  source 1..19: mol_type = other RNA
agatgtgtctgctacagaa

SEQ ID NO: 19 - RNA, 19 nt, synthetic construct
  source 1..19: mol_type = other RNA
gagcctgccagatgtgtct

SEQ ID NO: 20 - RNA, 19 nt, synthetic construct
  source 1..19: mol_type = other RNA
gagataaggtgtttgtcca

SEQ ID NO: 21 - RNA, 19 nt, synthetic construct
  source 1..19: mol_type = other RNA
ctcggagataaggtgttta

SEQ ID NO: 22 - RNA, 19 nt, synthetic construct
  source 1..19: mol_type = other RNA
aggactcggagataaggta

SEQ ID NO: 23 - RNA, 19 nt, synthetic construct
  source 1..19: mol_type = other RNA
aggaggactcggagataaa

SEQ ID NO: 24 - RNA, 19 nt, synthetic construct
  source 1..19: mol_type = other RNA
tcatcagcctggtggacaa

SEQ ID NO: 25 - RNA, 19 nt, synthetic construct
  source 1..19: mol_type = other RNA
tagtggtgctggacgtcat

SEQ ID NO: 26 - RNA, 19 nt, synthetic construct
  source 1..19: mol_type = other RNA
atggaagagaagcagatca

SEQ ID NO: 27 - RNA, 19 nt, synthetic construct
  source 1..19: mol_type = other RNA
gcctcatggaagagaagca

SEQ ID NO: 28 - RNA, 19 nt, synthetic construct
  source 1..19: mol_type = other RNA
ggagtagcctcatggaaga

SEQ ID NO: 29 - RNA, 19 nt, synthetic construct
  source 1..19: mol_type = other RNA
tgacaagcgaggaaactaa

SEQ ID NO: 30 - RNA, 19 nt, synthetic construct
  source 1..19: mol_type = other RNA
tcagctgtgagtccatcta

SEQ ID NO: 31 - RNA, 19 nt, synthetic construct
  source 1..19: mol_type = other RNA
gcattctcgagatcgctta

SEQ ID NO: 32 - RNA, 19 nt, synthetic construct
  source 1..19: mol_type = other RNA
tttgcattctcgagatcga

SEQ ID NO: 33 - RNA, 21 nt, synthetic construct
  source 1..21: mol_type = other RNA
gcaggaagcactgagattcgt

SEQ ID NO: 34 - RNA, 21 nt, synthetic construct
  source 1..21: mol_type = other RNA
atgtggatccacttgaactgg

SEQ ID NO: 35 - RNA, 21 nt, synthetic construct
  source 1..21: mol_type = other RNA
tttgctctgaggctctgcatc

SEQ ID NO: 36 - RNA, 21 nt, synthetic construct
  source 1..21: mol_type = other RNA
tctcagtgcttcctgcacgct

SEQ ID NO: 37 - RNA, 21 nt, synthetic construct
  source 1..21: mol_type = other RNA
aaagcatccgagtggagcaat

SEQ ID NO: 38 - RNA, 21 nt, synthetic construct
  source 1..21: mol_type = other RNA
aagcatccgagtggagcaatt

SEQ ID NO: 39 - RNA, 21 nt, synthetic construct
  source 1..21: mol_type = other RNA
tagtggagcaatttgccatca

SEQ ID NO: 40 - RNA, 21 nt, synthetic construct
  source 1..21: mol_type = other RNA
agcatcttcacctgctccgat

SEQ ID NO: 41 - RNA, 21 nt, synthetic construct
  source 1..21: mol_type = other RNA
atcttcacctgctccgatgcg

SEQ ID NO: 42 - RNA, 21 nt, synthetic construct
  source 1..21: mol_type = other RNA
atccacttgaactgggtcaga

SEQ ID NO: 43 - RNA, 21 nt, synthetic construct
  source 1..21: mol_type = other RNA
tccacttgaactgggtcagat

SEQ ID NO: 44 - RNA, 21 nt, synthetic construct
  source 1..21: mol_type = other RNA
tacttgaactgggtcagatca

SEQ ID NO: 45 - RNA, 21 nt, synthetic construct
  source 1..21: mol_type = other RNA
ttgaactgggtcagatcaacc

SEQ ID NO: 46 - RNA, 21 nt, synthetic construct
  source 1..21: mol_type = other RNA
tgaactgggtcagatcaacct

SEQ ID NO: 47 - RNA, 21 nt, synthetic construct
  source 1..21: mol_type = other RNA
ttctcaaagtctgtagcagac

SEQ ID NO: 48 - RNA, 21 nt, synthetic construct
  source 1..21: mol_type = other RNA
tctcaaagtctgtagcagaca

SEQ ID NO: 49 - RNA, 21 nt, synthetic construct
  source 1..21: mol_type = other RNA
tcaaagtctgtagcagacaca

SEQ ID NO: 50 - RNA, 21 nt, synthetic construct
  source 1..21: mol_type = other RNA
taaagtctgtagcagacacat

SEQ ID NO: 51 - RNA, 21 nt, synthetic construct
  source 1..21: mol_type = other RNA
ttctgtagcagacacatctgg

SEQ ID NO: 52 - RNA, 21 nt, synthetic construct
  source 1..21: mol_type = other RNA
agacacatctggcaggctcgt

SEQ ID NO: 53 - RNA, 21 nt, synthetic construct
  source 1..21: mol_type = other RNA
tggacaaacaccttatctccg

SEQ ID NO: 54 - RNA, 21 nt, synthetic construct
  source 1..21: mol_type = other RNA
taaacaccttatctccgagtc

SEQ ID NO: 55 - RNA, 21 nt, synthetic construct
  source 1..21: mol_type = other RNA
taccttatctccgagtccttt

SEQ ID NO: 56 - RNA, 21 nt, synthetic construct
  source 1..21: mol_type = other RNA
tttatctccgagtcctcctta

SEQ ID NO: 57 - RNA, 21 nt, synthetic construct
  source 1..21: mol_type = other RNA
ttgtccaccaggctgatgacg

SEQ ID NO: 58 - RNA, 21 nt, synthetic construct
  source 1..21: mol_type = other RNA
atgacgtccagcaccactagc

SEQ ID NO: 59 - RNA, 21 nt, synthetic construct
  source 1..21: mol_type = other RNA
tgatctgcttctcttccatga

SEQ ID NO: 60 - RNA, 21 nt, synthetic construct
  source 1..21: mol_type = other RNA
tgcttctcttccatgaggcta

SEQ ID NO: 61 - RNA, 21 nt, synthetic construct
  source 1..21: mol_type = other RNA
tcttccatgaggctactccca

SEQ ID NO: 62 - RNA, 21 nt, synthetic construct
  source 1..21: mol_type = other RNA
ttagtttcctcgcttgtcaga

SEQ ID NO: 63 - RNA, 21 nt, synthetic construct
  source 1..21: mol_type = other RNA
tagatggactcacagctgatg

SEQ ID NO: 64 - RNA, 21 nt, synthetic construct
  source 1..21: mol_type = other RNA
taagcgatctcgagaatgcaa

SEQ ID NO: 65 - RNA, 21 nt, synthetic construct
  source 1..21: mol_type = other RNA
tcgatctcgagaatgcaaaga

SEQ ID NO: 66 - RNA, 23 nt, synthetic construct
  source 1..23: mol_type = other RNA
acgaatctcagtgcttcctgcac

SEQ ID NO: 67 - RNA, 19 nt, synthetic construct
  source 1..19: mol_type = other RNA
ggtgtttgtcagcaaagat

SEQ ID NO: 68 - RNA, 19 nt, synthetic construct
  source 1..19: mol_type = other RNA
agttcaagtggatccacat

SEQ ID NO: 69 - RNA, 19 nt, synthetic construct
  source 1..19: mol_type = other RNA
ctgacccagttcaagtgga

SEQ ID NO: 70 - RNA, 19 nt, synthetic construct
  source 1..19: mol_type = other RNA
gagcctgccagatgtgtct

SEQ ID NO: 71 - RNA, 19 nt, synthetic construct
  source 1..19: mol_type = other RNA
gcctcatggaagagaagca

SEQ ID NO: 72 - RNA, 19 nt, synthetic construct
  source 1..19: mol_type = other RNA
ctgacccagttcaagtgga

SEQ ID NO: 73 - RNA, 19 nt, synthetic construct
  source 1..19: mol_type = other RNA
ctgacccagttcaagtgga

SEQ ID NO: 74 - RNA, 19 nt, synthetic construct
  source 1..19: mol_type = other RNA
ctgacccagttcaagtgga

SEQ ID NO: 75 - RNA, 19 nt, synthetic construct
  source 1..19: mol_type = other RNA
ctgacccagttcaagtgga

SEQ ID NO: 76 - RNA, 19 nt, synthetic construct
  source 1..19: mol_type = other RNA
ctgacccagttcaagtgga

SEQ ID NO: 77 - RNA, 19 nt, synthetic construct
  source 1..19: mol_type = other RNA
ctgacccagttcaagtgga

SEQ ID NO: 78 - RNA, 19 nt, synthetic construct
  source 1..19: mol_type = other RNA
ctgacccagttcaagtgga

SEQ ID NO: 79 - RNA, 19 nt, synthetic construct
  source 1..19: mol_type = other RNA
ctgacccagttcaattgga

SEQ ID NO: 80 - RNA, 19 nt, synthetic construct
  source 1..19: mol_type = other RNA
ctgacccagttcaagtgga

SEQ ID NO: 81 - RNA, 19 nt, synthetic construct
  source 1..19: mol_type = other RNA
ctgacccagttcaagtgga

SEQ ID NO: 82 - RNA, 19 nt, synthetic construct
  source 1..19: mol_type = other RNA
gagcctgccagatgtgtct

SEQ ID NO: 83 - RNA, 19 nt, synthetic construct
  source 1..19: mol_type = other RNA
gagcctgccagatgtgtct

SEQ ID NO: 84 - RNA, 19 nt, synthetic construct
  source 1..19: mol_type = other RNA
gagcctgccagatgtgtct

SEQ ID NO: 85 - RNA, 19 nt, synthetic construct
  source 1..19: mol_type = other RNA
gagcctgccagatgtgtct

SEQ ID NO: 86 - RNA, 19 nt, synthetic construct
  source 1..19: mol_type = other RNA
gagcctgccagatgtgtct

SEQ ID NO: 87 - RNA, 19 nt, synthetic construct
  source 1..19: mol_type = other RNA
agttcaagtggatccacat

SEQ ID NO: 88 - RNA, 19 nt, synthetic construct
  source 1..19: mol_type = other RNA
agttcaagtggatccacat

SEQ ID NO: 89 - RNA, 19 nt, synthetic construct
  source 1..19: mol_type = other RNA
tgcagagcctcagagcaaa

SEQ ID NO: 90 - RNA, 19 nt, synthetic construct
  source 1..19: mol_type = other RNA
cgtgcaggaagcactgaga

SEQ ID NO: 91 - RNA, 19 nt, synthetic construct
  source 1..19: mol_type = other RNA
cggagcaggtgaagatgct

SEQ ID NO: 92 - RNA, 19 nt, synthetic construct
  source 1..19: mol_type = other RNA
atctgacccagttcaagta

SEQ ID NO: 93 - RNA, 19 nt, synthetic construct
  source 1..19: mol_type = other RNA
gtgtctgctacagacttta

SEQ ID NO: 94 - RNA, 19 nt, synthetic construct
  source 1..19: mol_type = other RNA
gagataaggtgtttgtcca

SEQ ID NO: 95 - RNA, 19 nt, synthetic construct
  source 1..19: mol_type = other RNA
tcatcagcctggtggacaa

SEQ ID NO: 96 - RNA, 19 nt, synthetic construct
  source 1..19: mol_type = other RNA
tgcagagcctcagagcaaa

SEQ ID NO: 97 - RNA, 19 nt, synthetic construct
  source 1..19: mol_type = other RNA
cgtgcaggaagcactgaga

SEQ ID NO: 98 - RNA, 19 nt, synthetic construct
  source 1..19: mol_type = other RNA
cggagcaggtgaagatgct

SEQ ID NO: 99 - RNA, 19 nt, synthetic construct
  source 1..19: mol_type = other RNA
atctgacccagttcaagta

SEQ ID NO: 100 - RNA, 19 nt, synthetic construct
  source 1..19: mol_type = other RNA
gtgtctgctacagacttta

SEQ ID NO: 101 - RNA, 19 nt, synthetic construct
  source 1..19: mol_type = other RNA
gagataaggtgtttgtcca

SEQ ID NO: 102 - RNA, 19 nt, synthetic construct
  source 1..19: mol_type = other RNA
tcatcagcctggtggacaa

SEQ ID NO: 103 - RNA, 21 nt, synthetic construct
  source 1..21: mol_type = other RNA
atctttgctgacaaacaccac

SEQ ID NO: 104 - RNA, 21 nt, synthetic construct
  source 1..21: mol_type = other RNA
atgtggatccacttgaactgg

SEQ ID NO: 105 - RNA, 21 nt, synthetic construct
  source 1..21: mol_type = other RNA
tccacttgaactgggtcagat

SEQ ID NO: 106 - RNA, 21 nt, synthetic construct
  source 1..21: mol_type = other RNA
agacacatctggcaggctcgt

SEQ ID NO: 107 - RNA, 21 nt, synthetic construct
  source 1..21: mol_type = other RNA
tgcttctcttccatgaggcta

SEQ ID NO: 108 - RNA, 21 nt, synthetic construct
  source 1..21: mol_type = other RNA
tccacttgaactgggtcagat

SEQ ID NO: 109 - RNA, 21 nt, synthetic construct
  source 1..21: mol_type = other RNA
tccacttgaactgggtcagat

SEQ ID NO: 110 - RNA, 21 nt, synthetic construct
  source 1..21: mol_type = other RNA
tccacttgaactgggtcagat

SEQ ID NO: 111 - RNA, 21 nt, synthetic construct
  source 1..21: mol_type = other RNA
tccacttgaactgggtcagat

SEQ ID NO: 112 - RNA, 21 nt, synthetic construct
  source 1..21: mol_type = other RNA
tccacttgaactgggtcagat

SEQ ID NO: 113 - RNA, 21 nt, synthetic construct
  source 1..21: mol_type = other RNA
tccacttgaactgggtcagat

SEQ ID NO: 114 - RNA, 21 nt, synthetic construct
  source 1..21: mol_type = other RNA
tccacttgaactgggtcagat

SEQ ID NO: 115 - RNA, 21 nt, synthetic construct
  source 1..21: mol_type = other RNA
tccacttgaactgggtcagtt

SEQ ID NO: 116 - RNA, 21 nt, synthetic construct
  source 1..21: mol_type = other RNA
tccacttgaactgggtcagat

SEQ ID NO: 117 - RNA, 21 nt, synthetic construct
  source 1..21: mol_type = other RNA
tccacttgaactgggtcagat

SEQ ID NO: 118 - RNA, 21 nt, synthetic construct
  source 1..21: mol_type = other RNA
tccaattgaactgggtcagat

SEQ ID NO: 119 - RNA, 21 nt, synthetic construct
  source 1..21: mol_type = other RNA
agacacatctggcaggctcgt

SEQ ID NO: 120 - RNA, 21 nt, synthetic construct
  source 1..21: mol_type = other RNA
agacacatctggcaggctcgt

SEQ ID NO: 121 - RNA, 21 nt, synthetic construct
  source 1..21: mol_type = other RNA
agacacatctggcaggctcgt

SEQ ID NO: 122 - RNA, 21 nt, synthetic construct
  source 1..21: mol_type = other RNA
atgtggatccacttgaactgg

SEQ ID NO: 123 - RNA, 21 nt, synthetic construct
  source 1..21: mol_type = other RNA
atgtggatccacttgaactgg

SEQ ID NO: 124 - RNA, 21 nt, synthetic construct
  source 1..21: mol_type = other RNA
tttgctctgaggctctgcatc

SEQ ID NO: 125 - RNA, 21 nt, synthetic construct
  source 1..21: mol_type = other RNA
tctcagtgcttcctgcacgct

SEQ ID NO: 126 - RNA, 21 nt, synthetic construct
  source 1..21: mol_type = other RNA
agcatcttcacctgctccgat

SEQ ID NO: 127 - RNA, 21 nt, synthetic construct
  source 1..21: mol_type = other RNA
tacttgaactgggtcagatca

SEQ ID NO: 128 - RNA, 21 nt, synthetic construct
  source 1..21: mol_type = other RNA
taaagtctgtagcagacacat

SEQ ID NO: 129 - RNA, 21 nt, synthetic construct
  source 1..21: mol_type = other RNA
tggacaaacaccttatctccg

SEQ ID NO: 130 - RNA, 21 nt, synthetic construct
  source 1..21: mol_type = other RNA
ttgtccaccaggctgatgacg

SEQ ID NO: 131 - RNA, 19 nt, synthetic construct
  source 1..19: mol_type = other RNA
ggtgtttgtcagcaaagat

SEQ ID NO: 132 - RNA, 19 nt, synthetic construct
  source 1..19: mol_type = other RNA
agttcaagtggatccacat

SEQ ID NO: 133 - RNA, 19 nt, synthetic construct
  source 1..19: mol_type = other RNA
ctgacccagttcaagtgga

SEQ ID NO: 134 - RNA, 19 nt, synthetic construct
  source 1..19: mol_type = other RNA
gagcctgccagatgtgtct

SEQ ID NO: 135 - RNA, 19 nt, synthetic construct
  source 1..19: mol_type = other RNA
gcctcatggaagagaagca

SEQ ID NO: 136 - RNA, 19 nt, synthetic construct
  source 1..19: mol_type = other RNA
ctgacccagttcaagtgga

SEQ ID NO: 137 - RNA, 19 nt, synthetic construct
  source 1..19: mol_type = other RNA
ctgacccagttcaagtgga

SEQ ID NO: 138 - RNA, 19 nt, synthetic construct
  source 1..19: mol_type = other RNA
ctgacccagttcaagtgga

SEQ ID NO: 139 - RNA, 19 nt, synthetic construct
  source 1..19: mol_type = other RNA
ctgacccagttcaagtgga

SEQ ID NO: 140 - RNA, 19 nt, synthetic construct
  source 1..19: mol_type = other RNA
ctgacccagttcaagtgga

SEQ ID NO: 141 - RNA, 19 nt, synthetic construct
  source 1..19: mol_type = other RNA
ctgacccagttcaagtgga

SEQ ID NO: 142 - RNA, 19 nt, synthetic construct
  source 1..19: mol_type = other RNA
ctgacccagttcaattgga

SEQ ID NO: 143 - RNA, 19 nt, synthetic construct
  source 1..19: mol_type = other RNA
gagcctgccagatgtgtct

SEQ ID NO: 144 - RNA, 19 nt, synthetic construct
  source 1..19: mol_type = other RNA
gagcctgccagatgtgtct

SEQ ID NO: 145 - RNA, 19 nt, synthetic construct
  source 1..19: mol_type = other RNA
gagcctgccagatgtgtct

SEQ ID NO: 146 - RNA, 19 nt, synthetic construct
  source 1..19: mol_type = other RNA
agttcaagtggatccacat

SEQ ID NO: 147 - RNA, 19 nt, synthetic construct
  source 1..19: mol_type = other RNA
tgcagagcctcagagcaaa

SEQ ID NO: 148 - RNA, 19 nt, synthetic construct
  source 1..19: mol_type = other RNA
cgtgcaggaagcactgaga

SEQ ID NO: 149 - RNA, 19 nt, synthetic construct
  source 1..19: mol_type = other RNA
cggagcaggtgaagatgct

SEQ ID NO: 150 - RNA, 19 nt, synthetic construct
  source 1..19: mol_type = other RNA
atctgacccagttcaagta

SEQ ID NO: 151 - RNA, 19 nt, synthetic construct
  source 1..19: mol_type = other RNA
gtgtctgctacagacttta

SEQ ID NO: 152 - RNA, 19 nt, synthetic construct
  source 1..19: mol_type = other RNA
gagataaggtgtttgtcca

SEQ ID NO: 153 - RNA, 19 nt, synthetic construct
  source 1..19: mol_type = other RNA
tcatcagcctggtggacaa